European Patent Application EP 4 219 560 A2, published August 2, 2023. Title: Integrin alph-V-beta-8 Neutralizing Antibody. Applicant: The Regents of the University of California. The sequence listing filed with the application follows.

SEQUENCE LISTING (12 sequences)

SEQ ID NO: 1 - protein, 116 aa, synthetic construct
  REGION 1..116: note = Synthetic peptide of engineered variable heavy region of clone 37E1 from Mus musculus
EVQLVESGGGLVQPGGSLNLSCAASGFVFSRYWMSWVRQAPGKGLEWIGEINPDSSTINYTSSLKDKFIISRDNAKNTLYLQMNKVRSEDTALYYCACLITTEDYWGQGTSVTVSS

SEQ ID NO: 2 - protein, 116 aa, synthetic construct
  REGION 1..116: note = Synthetic peptide of engineered variable heavy region of clone 37E1b5 from Mus musculus
EVQLVESGGGLVQPGGSLNLSCAVSGFVFSRYWMSWVRQAPGKGLEWIGEINPDSSTINYTSSLKDKFIISRDNAKNTLYLQMNKVRSEDTALYYCACLITTEDYWGQGTSVTVSS

SEQ ID NO: 3 - protein, 108 aa, synthetic construct
  REGION 1..108: note = Synthetic peptide of engineered variable light region of clone 37E1 from Mus musculus
QIVLTQSPSSMYASLGERVTIPCKASQDINSYLSWFQQKPGKSPKTLIYRANRLVDGVPSRFSGSGSGQDYSLTISSLEYEDMGIYYCLQYDEFPYTFGGGTKLEIKA

SEQ ID NO: 4 - protein, 108 aa, synthetic construct
  REGION 1..108: note = Synthetic peptide of engineered variable light region of clone 37E1B5 from Mus musculus
QIVLTQSPSSMYASLGERVTIPCKASQDINSYLSWFQQKPGKSPKTLIYYANRLVDGVPSRFSGSGSGQDYSLTISSLEYEDMGIYYCLQYDEFPYTFGGGTKLEIKA

SEQ ID NO: 5 - protein, 5 aa, synthetic construct
  REGION 1..5: note = Synthetic peptide of CDR1 of engineered variable heavy region of Mus musculus clone 37E1 or 37E1b5
RYWMS

SEQ ID NO: 6 - protein, 17 aa, synthetic construct
  REGION 1..17: note = Synthetic peptide of CDR2 of engineered variable heavy region of Mus musculus clone 37E1 or 37E1b5
EINPDSSTINYTSSLKD

SEQ ID NO: 7 - protein, 7 aa, synthetic construct
  REGION 1..7: note = Synthetic peptide of CDR3 of engineered variable heavy region of Mus musculus clone 37E1 or 37E1b5
LITTEDY

SEQ ID NO: 8 - protein, 11 aa, synthetic construct
  REGION 1..11: note = Synthetic peptide of CDR1 of engineered variable light region of Mus musculus clone 37E1 or 37E1b5
KASQDINSYLS

SEQ ID NO: 9 - protein, 7 aa, synthetic construct
  REGION 1..7: note = Synthetic peptide of CDR2 of engineered variable light region of Mus musculus clone 37E1 or 37E1b5
  VARIANT 1: note = X can be Arg or Tyr
XANRLVD

SEQ ID NO: 10 - protein, 9 aa, synthetic construct
  REGION 1..9: note = Synthetic peptide of CDR3 of engineered variable light region of Mus musculus clone 37E1 or 37E1b5
LQYDEFPYT

SEQ ID NO: 11 - protein, 107 aa, Homo sapiens
ISGGSRSERCDIVSNLISKGCSVDSIEYPSVHVIIPTENEINTQVTPGEVSIQLRPGAEANFMLKVHPLKKYPVDLYYLVDVSASMHNNIEKLNSVGNDLSRKMAFF

SEQ ID NO: 12 - protein, 107 aa, Mus musculus
VSGGSGSERCDTVSSLISKGCPVDSIEYLSVHVVTSSENEINTQVTPGEVSVQLHPGAEANFMLKVRPLKKYPVDLYYLVDVSASMHNNIEKLNSVGNDLSKKMALY